European Patent Application EP 4 729 605 A1, published April 22, 2026. Title: Crotyl alcohol-producing Hydrogenophilus bacterium transformant. Applicant: 株式会社ＣＯ２資源化研究所. The sequence listing filed with the application follows.

SEQUENCE LISTING (58 sequences)

SEQ ID NO: 1 - DNA, 2601 bp, Clostridium akagii
  source 1..2601: mol_type = genomic DNA
atgaaagtaacaaacatagaagagttaaatataaagctcaaaagtgtaaaagaagctcaaaaagagttttcaacctttacccaggagatggttgatgaaatctttaaaagagtagcaattgcagcattagaagccagaataccattggctaaaatggctgtggaagaaagtggtatgggattactagaggataaggtaataaaaaaccattttgctgctgaatatatatataataaatataaggatgaaaaaacatgtggtgttattgaaagagatgaaacctatggtataacaaaaatagcagagccaataggtgttgtagcagctatagtaccaactaccaatcctacctctacagtgatttttaaaacactaatctccttaaaaactagaaatggcataatattttctcctcatccaagagcaaaaaaatcaacagtagcagctgcaaaaataatgttagaggctgcagttaaggctggggcacctgagggaataatagggtggatagacgaaccttctatagaactttcaaaaatattaatgagtgaagcagatgtaatactagctacaggaggacctagtatggttaaatcggcttattcatctggtaaaccagctattggagttggacctgggaatacaccgtctataatagatgaaagtgcagatatacaaatggccgtaagttcaataatattatctaaaacttatgataatggtgtaatatgtgcttcggaacaatctgtaatagtcttagattccatatataataaggttaaaaatgaattcattaaacgaggagcttatatattaagtaaaaatgagatagaaaaagttaaaatgataatgtttaataatgggaatataaatgctagtgtagttggacaatcagcttgcaaaatagctaagttggcagatattaatgtacctgaatggacaaaggtacttattggagaagttaagtctgtggaattagaagaactattttcacatgaaaaattatccacagtattagctatgtatagagtaaatagttttgatgaagctttagaaaaggccgaaagactggtggaattaggtggaaaaggacatacatcatcattgtttatagattctgtatgtgaaaaagaaaaaatagaaaagtttagttttaaaatgaaaactgtaagaacctttataaatataccttcatcccaaggggctagtggtgatttattcaattttaaaatagcaccttcctttactttaggttgtggattctggggtggaaattcagtgtctgaaaacgtaggacctaaacatttgttgaatataaaaacagtagctgagagaagggaaaatatgctttggtttaaggtaccagaaaaaatatacttcaaatatggatgtttggaatttgcacttagggaattaaaagatatgggtaagaaaaaagcatttattgtaactgataaagtgctttatgaattaggatatgccgataaagtaacgaaagttttagaaaaaatggacatacggtttaaagttttttcagatgttgagccagaccctacacttgcctgtgcgagtaaaggcgccaaagaaatgcttgaatttgaaccagacactataatatccataggtggaggatcagctatggatgcggctaaaattatgcaagttttatatgagcatccagaagagaagtttgatgaactggcactgaaatttatggatataagaaagcgaatacacagttttccaaagcttggaattaaggctatatcagtagcaataccaacaactgctggtactggttcagaagtaacaccttttgcagtaataacagatgaaaaaacggggatgaaatatccactttcagattatgagttaacaccgaatgtggcaattgtagatgcagaatttatgatgaatatgcctaagggtctaactgcggcaacagggatagatgcactaactcatgctattgaagcctatgtatctgttatggcaacggaatacacagatggattggcacttcaagcaataaaaatgatatttgaatatttaccagcagcatataatgaaggaaagactaatatagttgctagagagaagatggcaaatgcatctacaatagcaggtatggcgttcggaaatgcatttttaggagtatgtcattcaatggcccataaattaggagcccagcaccatgtaccccatggtattgctaatgcagtgttaattgaggaagtaattagatttaatgcagtagacaatccagtaagacaaacttcatttccacaatataaatatccagatgcaaaagaaagatatgctaggattgctgattatttaaaactaagtggaaatacagatagtgacaaagtagaacaactaataaaggcaattactaatttaaaaataaaattaagtattccattgactataaaggatgcaggaattaaagaagaagctttttatttaacattggatgatatgtctgagaaggcttttgatgatcaatgcactagcgctaatcctagatatccattgataagcgaaattaaacaaatgtttataaacgcatttggtgaaattaaaatgggagaaaaataa

SEQ ID NO: 2 - protein, 866 aa, Clostridium akagii
MKVTNIEELNIKLKSVKEAQKEFSTFTQEMVDEIFKRVAIAALEARIPLAKMAVEESGMGLLEDKVIKNHFAAEYIYNKYKDEKTCGVIERDETYGITKIAEPIGVVAAIVPTTNPTSTVIFKTLISLKTRNGIIFSPHPRAKKSTVAAAKIMLEAAVKAGAPEGIIGWIDEPSIELSKILMSEADVILATGGPSMVKSAYSSGKPAIGVGPGNTPSIIDESADIQMAVSSIILSKTYDNGVICASEQSVIVLDSIYNKVKNEFIKRGAYILSKNEIEKVKMIMFNNGNINASVVGQSACKIAKLADINVPEWTKVLIGEVKSVELEELFSHEKLSTVLAMYRVNSFDEALEKAERLVELGGKGHTSSLFIDSVCEKEKIEKFSFKMKTVRTFINIPSSQGASGDLFNFKIAPSFTLGCGFWGGNSVSENVGPKHLLNIKTVAERRENMLWFKVPEKIYFKYGCLEFALRELKDMGKKKAFIVTDKVLYELGYADKVTKVLEKMDIRFKVFSDVEPDPTLACASKGAKEMLEFEPDTIISIGGGSAMDAAKIMQVLYEHPEEKFDELALKFMDIRKRIHSFPKLGIKAISVAIPTTAGTGSEVTPFAVITDEKTGMKYPLSDYELTPNVAIVDAEFMMNMPKGLTAATGIDALTHAIEAYVSVMATEYTDGLALQAIKMIFEYLPAAYNEGKTNIVAREKMANASTIAGMAFGNAFLGVCHSMAHKLGAQHHVPHGIANAVLIEEVIRFNAVDNPVRQTSFPQYKYPDAKERYARIADYLKLSGNTDSDKVEQLIKAITNLKIKLSIPLTIKDAGIKEEAFYLTLDDMSEKAFDDQCTSANPRYPLISEIKQMFINAFGEIKMGEK

SEQ ID NO: 3 - DNA, 1023 bp, Bacillus coagulans
  source 1..1023: mol_type = genomic DNA
atgagagcagcagtcgtcagttctgataagcaaaaactggtagaggtcaaagatgtgcagttgcgtccacttgaatatggggaagctttggtggatatcgaatactgcggtgtctgccatacggatctgcatgtggcaaagggcgactttggcgatgtgccgggacgcattctcggccatgaaggagtcggcattgtcagggaagtcgcggatggtgtcacttctcttaaagtgggagatcgtgtaagcgttgcctggttttttgaaggctgcgggcattgtgagtactgtttaacgggaaatgaaacattttgccgtgatgtgaaaaatgcaggctacagtgtcgacggagcaatggcagagcagtgcatcgtcaaagcggattacgccgtaaaagtgccggaagggctggatccaaggcaggcgacgagcattacttgcgcaggtgtcaccacttataaagccattaaagtcgcagatgtgaagccgggcgaatggattgccatttatggagccggcggtcttggtaaccttgctgtccagtacgccaaacatgtatttaatgcgaaagtcattgcgatcgatatcaatgacgacaaactttcactggcaaaagaagtcggtgctgatctcacctttaattccaaaatgaaaggcgatccggctgaatggatccaaaaagaagttggcggcgcgcatgctgcagtggtaacggctgtttcaaaacaggcttttaaccaggctgtccactctgtacggccggtttcaaaagtcgttgctgtcgggctccctccggaaacaatggatcttgaaattgtgaagacggttcttgacggaatagaagtcgtcggctctttggtaggcacgagaaaagaccttgaggaagcctttatgttcggggcggaaggaaaagtcgtcccggttgtgcacacgcgcagactggaagaagtgggagatgtgtttaaagaaatggaagaaggcagaatacagggcaggatggtcctggatatgtcgttgaaataa

SEQ ID NO: 4 - protein, 340 aa, Bacillus coagulans
MRAAVVSSDKQKLVEVKDVQLRPLEYGEALVDIEYCGVCHTDLHVAKGDFGDVPGRILGHEGVGIVREVADGVTSLKVGDRVSVAWFFEGCGHCEYCLTGNETFCRDVKNAGYSVDGAMAEQCIVKADYAVKVPEGLDPRQATSITCAGVTTYKAIKVADVKPGEWIAIYGAGGLGNLAVQYAKHVFNAKVIAIDINDDKLSLAKEVGADLTFNSKMKGDPAEWIQKEVGGAHAAVVTAVSKQAFNQAVHSVRPVSKVVAVGLPPETMDLEIVKTVLDGIEVVGSLVGTRKDLEEAFMFGAEGKVVPVVHTRRLEEVGDVFKEMEEGRIQGRMVLDMSLK

SEQ ID NO: 5 - DNA, 1014 bp, Zymomonas mobillis subsp.pomaseae
  source 1..1014: mol_type = genomic DNA
atgaaagcagccgtcataactaaagatcatacgatcgaagtgaaagacaccaaattacgccctctgaaatacggggaagcgcttttggaaatggaatattgcggggtatgtcataccgatctccacgtgaaaaacggggattttggcgatgaaaccggcagaattaccggccatgaaggcatcggtatcgtcaagcaggtcggggaaggggttacttctctgaaagtcggtgaccgcgccagtgttgcatggttcttcaaaggctgcggccattgcgagtattgtgtcagcgggaatgaaacgctttgccgcaacgttgaaaatgccggttatacggttgacggcgctatggcagaagaatgcatcgtcgttgccgattactcggtcaaagtgccagatggtcttgatcctgcggttgccagcagcatcacttgcgcgggtgtaaccacctataaagcagtcaaagtttctcagatacagccgggacaatggctggctatctatggcttgggcggtttaggcaatctagcccttcaatatgccaagaatgttttcaacgccaaagtgatcgcgatcgatgtcaatgatgaacagctcgcttttgccaaagagctgggcgcagatatggtcatcaatccgaaaaacgaagatgctgccaaaatcattcaggaaaaagtcggcggcgcacatgcgacggtggtgacggctgttgccaaatccgcctttaactcggctgttgaggctatccgcgcgggtggccgtgttgtcgccgttggtctgcctcctgaaaaaatggatttgagcattcctcgtttggtgcttgacggtatcgaagtcctaggttccttggtcggaacgcgggaagatttgaaagaagccttccagtttgcagccgaaggtaaggtcaaaccgaaagtcaccaagcgtaaagtcgaagaaatcaaccaaatctttgacgaaatggaacatggtaaattcacaggccgtatggttgttgattttacccatcactag

SEQ ID NO: 6 - protein, 337 aa, Zymomonas mobillis subsp.pomaseae
MKAAVITKDHTIEVKDTKLRPLKYGEALLEMEYCGVCHTDLHVKNGDFGDETGRITGHEGIGIVKQVGEGVTSLKVGDRASVAWFFKGCGHCEYCVSGNETLCRNVENAGYTVDGAMAEECIVVADYSVKVPDGLDPAVASSITCAGVTTYKAVKVSQIQPGQWLAIYGLGGLGNLALQYAKNVFNAKVIAIDVNDEQLAFAKELGADMVINPKNEDAAKIIQEKVGGAHATVVTAVAKSAFNSAVEAIRAGGRVVAVGLPPEKMDLSIPRLVLDGIEVLGSLVGTREDLKEAFQFAAEGKVKPKVTKRKVEEINQIFDEMEHGKFTGRMVVDFTHH

SEQ ID NO: 7 - DNA, 2718 bp, Thermoclostridium caenicola
  source 1..2718: mol_type = genomic DNA
atggaaaacaaagaaagaaagattgtagacagtgtggacgcgttaaagaaagtcattgcccgggtaagggaagcgcaaaggaaattttcaacctattcccaggaacaggtggatgaaatttttaaggctgctgccactgccgcaaaccaggcaagaattccgctggcgaaaatggcggtggaagaaaccggtatgggcgttgtggaagataaagttataaaaaaccactatgccgccgaatatgtttacaatacgtataagaacgtaagaacctgcggggttttggaagaagataaggcatacggtatcaaaaaaattgccgagcctgtcggtgtgattgccgctgttattcctaccactaaccctacttccacggcaatttttaaaaccctgatcgcgctgaaaacacgcaatgccgttattatcagcccacatccgagagctaaaaaatgcaccatcgctgcggcaaaaatcgtattggatgctgccgttgccgcgggggctccggaagggattattgactggattgatgtgccgaacattgagttgaccaatctgcttatgaaagaagcagacattatccttgccacaggtggtcccggtatggtgaaggcggcttattcctccgggaaaccggctatcggtgtcgggcctggcaatactccggccgttattgatgaaagcgccgacgttgtccttgccgtgaactccattattcattccaaaacgtttgataatggtatgatttgcgcatcagaacaatcggtaattgttcacaagaatgtttatgacgctgtaaaagctgaatttgcggcccgtggatgctatttccttaaagaagatgaaattgaaaaggtacgcaagacgatttttgtcaacggcgcgttaaatgcccagattgttggtcagccggcatacaaaattgccgaacttgccggtgtgaaagtgcctgtaggcacaaaaatcctcatcggagaagttgacagcacagacccgtcggaagaatttgcccatgaaaagctgtcacctgtccttgcgatgtataaagctgaggatattcatgacgcttttgagaaagccgaacgtttggttgccaacggaggttacggtcataccgcagcaatttatttggatgtaaccaccgaacaggctaaaattgacgaattcgcttcgcgtttgaagacctgccgtatacttgtgaatactccgtcttctcagggagctatcggcgacatttacaactttaagcttgcgccgtcgttaactcttggctgtggttcctggggcggaaattcggtttccgaaaatgttggggtaaaacacctgcttaatatcaaaacggttgttgaaagaagggaaaatatgctgtggttccgcgctcccgaaaaaatatacatcaaaaagggatgtttgccggtagcccttaatgagttgaaatacgtcatgggtaagaaacgcgcttttatagttaccgacagcttcctctatcacaatggttacacaaagcccattaccgacagacttgacgaactgggcattgaacatacaacgttttttgatgttttacccgatccgacgctttcctgcgcaaaagcgggagctgagcagatgagagccttccagcccgataccattattgccttcggtggcggatctgcgatggacgccgcgaaaatcatgtgggtaatgtatgagcatcccgaagttgatttcatggacatggctatgcgttttatggatatcaggaaaagggtttatacatttccgaaaatgggagaaaaggcgtattttgttgcaataccgacttctgcgggtaccggatccgaagtaactccttttgcggttatcaccgacgaaaagagtggagtaaaatatcccctcgcagactacgagttgctccccgacatggcaattatagatgtggattttcacatgagtgctcccaagggccttaccgccgcagcaggtatagatgccctcacccatgcgcttgaggcgtacgtttctcttatggccactgattttaccgacggactggcgaaacaggctctgcagatgatttttaaatacctgccccgcgcctatgataacggtcagaccgatgtggaagcacgtgaaaaaatggctaatgccgccaccattgcaggtatggcgtttgcaaatgctttccttggtgtttgccattccatggcacataagctgggcgctttttatcatttgcctcatggtattgccaacgcgcttatgatagaagaagtaatccgtttcaacgcttcggaagcaccggccaaaatgggaactttcccgcaatacggatacccgcacgctttaagacgttatgccgaaattgctgaggcgcttaatctcggcggcgaaaacgatcatgaaaagctggaaaatctcattaaagccattaatgatctgaaggcaagggtggggatcaagtcatcaatcaaagagtatggcataaatgagaaggaattcctggaacgcctcgacgagatggttgaacaggcattcgacgaccagtgcaccggtaccaatccgcgatatccgctgatgagcgaaataaggcaaatgtatctgaatgcttattacggcaaaaaacattttgtcgatgaagaaaagccaaatgaagcggatatcgccgggacagaggatgaaaacaaagttaaaaaggcgtatctgagagccagagtcggagcgaagagagcatga

SEQ ID NO: 8 - protein, 905 aa, Thermoclostridium caenicola
MENKERKIVDSVDALKKVIARVREAQRKFSTYSQEQVDEIFKAAATAANQARIPLAKMAVEETGMGVVEDKVIKNHYAAEYVYNTYKNVRTCGVLEEDKAYGIKKIAEPVGVIAAVIPTTNPTSTAIFKTLIALKTRNAVIISPHPRAKKCTIAAAKIVLDAAVAAGAPEGIIDWIDVPNIELTNLLMKEADIILATGGPGMVKAAYSSGKPAIGVGPGNTPAVIDESADVVLAVNSIIHSKTFDNGMICASEQSVIVHKNVYDAVKAEFAARGCYFLKEDEIEKVRKTIFVNGALNAQIVGQPAYKIAELAGVKVPVGTKILIGEVDSTDPSEEFAHEKLSPVLAMYKAEDIHDAFEKAERLVANGGYGHTAAIYLDVTTEQAKIDEFASRLKTCRILVNTPSSQGAIGDIYNFKLAPSLTLGCGSWGGNSVSENVGVKHLLNIKTVVERRENMLWFRAPEKIYIKKGCLPVALNELKYVMGKKRAFIVTDSFLYHNGYTKPITDRLDELGIEHTTFFDVLPDPTLSCAKAGAEQMRAFQPDTIIAFGGGSAMDAAKIMWVMYEHPEVDFMDMAMRFMDIRKRVYTFPKMGEKAYFVAIPTSAGTGSEVTPFAVITDEKSGVKYPLADYELLPDMAIIDVDFHMSAPKGLTAAAGIDALTHALEAYVSLMATDFTDGLAKQALQMIFKYLPRAYDNGQTDVEAREKMANAATIAGMAFANAFLGVCHSMAHKLGAFYHLPHGIANALMIEEVIRFNASEAPAKMGTFPQYGYPHALRRYAEIAEALNLGGENDHEKLENLIKAINDLKARVGIKSSIKEYGINEKEFLERLDEMVEQAFDDQCTGTNPRYPLMSEIRQMYLNAYYGKKHFVDEEKPNEADIAGTEDENKVKKAYLRARVGAKRA

SEQ ID NO: 9 - DNA, 2619 bp, Thermoanaerobacter mathranii
  source 1..2619: mol_type = genomic DNA
atgcctactttattacaagaaaaaaaggaaacaaaagaaaaaacagaagtaaaagaaacaacagatgttaaaaaacaaatagacctattagtagaaagggcaaaaagagcccaagaaaaattcatgtcatacactcaagagcaaattgatgaaatagtcaaagttatggcactagcgggcatagaaaagcatgtagaactggcaaaattagctcatgaagaaacgaaaatgggggtttatgaagacaaaataacgaaaaatctctttgcagtagaatatgtgtacaattatataaaagacaaaaagactgtcggcatccttagtgaaaacttagaagaaaatcatatggaagtggcagagcctgtaggaattatagcaggggttacccccgtgacaaaccctacctctacaacaatgtttaaatgcttaatagctatcaaaacaagaaatccaataatttttagtttccatcccaaagcattaaaatgtagtatagaagcagcaaagaccatgtacgaggcagcattaaaggcgggtgctcccgaaggatgcataggttggattgaaacaccttcaattgaagcaacgcaacttctcatgacacaccccggcgtctcccttatcctcgcaacaggcggtgcgggaatggtaaaagctgcttacagctcaggaaaacccgcccttggcgtaggtcctggcaatgtcccctgctacattgaaaaaactgcaaatattaaaagagcggtctcagacctaatacttagcaaaacttttgacaatggcacagtatgcgcatcagaacaagctgtgataatagatgaagaaatagccaatgaagtaaaaaaattaatgagagaatatggttgctatttcttaaataaagaagaaactaaaaagttagaagaattcgctatagacaaaaacaccggtttaatgaatccagcagttgtgggtcagcctgcagtgaaaattgctcaaatggctggatttaaagttcctgaaaataccaaaatacttgtagctgaatatccagctgtaggtcctaaatatcctctatccagagaaaaactaagcccaatacttgctttatacacagtcaaagattacaaagaaggtataaaaagatgcgaagaaatgatacaattcggcggacttggtcactctgcggtaatacattctgaaaaccaacaaattattaatgaatttgcaaatagagtacaagcaagtagaatccttgtaaacgcccctgcttcacaaggcgctattggagacatttataacacggctactccatctttgactttgggttgcggtacaatgggtggaaattcaacaacagataatgtaagtgtttataaccttataaacataaaacgagtttttataagaaaagagagaatgaaatggttcagagttccaccacaaatctattttgaaagagggtcaatacagtatctatcacaagtaaaaggcaaaaaagcttttattgtaacagaccctgcaatggttaaattaggttttgtagataaagtgacatatcaattagataaagcaaatattaaatatgaaattttctctgaagtagaaccagacccatcagttgacactgtagaaaaagggataaaaataatgaaggagttcgagcctgacttactaatagctgtaggtggtggttctgcaatagacgcagcaaagggaatgtggcttttttatgagtaccctgacacaaaatttgaagacttaaggttaaagttcatggacataagaaaaagaacttatagatttcctgaactcggcaaaaaagctttatttatcgcaataccaaccaccagcggtacaggttctgaagtcacagcctttgcagttataacagacaaaaagaaaaatataaagtaccctcttacagattacgaattgacaccagatattgctataatagaccctgactttgtcatgacaattccaccctctgtaactgcagatacaggtatggatgctttaactcatgccattgaagcttatgtatccgtgatggcatcagactatacagacgccctcgcagaaaaagccataaaactgatatttgaatatctccctaaagcatataaaaacggacaagacaaagtcgcccgcgaaaagatgcacaatgcttcttgcatagcaggaatggcattcacaaatgcatttttaggaataaaccacagtatggcccacatacttggcgctaaattccaccttccccatggaagggcaaatgcgatacttctgccctatgtcatagaatacaatgctgagttacctaaaaaatttgcctcattcccacaatatgaatatcccaaagcagccgagaaatacgcagaaattgcaaaattcttaggacttcctgcatcaaccactgatgaaggagtaaaaagtctcattgaagcaataaaaaatctcatgaaagagttaaatcttcctcttacacttaaagatgcgggaataaacaaagaagaatttgaaaaacaaataatggaaatggctgatatagccttcaacgaccagtgcaccggttcaaatccaagaatgccattggtatcagaaattgcagaaatatatagaaaagcctatggagaataa

SEQ ID NO: 10 - protein, 872 aa, Thermoanaerobacter mathranii
MPTLLQEKKETKEKTEVKETTDVKKQIDLLVERAKRAQEKFMSYTQEQIDEIVKVMALAGIEKHVELAKLAHEETKMGVYEDKITKNLFAVEYVYNYIKDKKTVGILSENLEENHMEVAEPVGIIAGVTPVTNPTSTTMFKCLIAIKTRNPIIFSFHPKALKCSIEAAKTMYEAALKAGAPEGCIGWIETPSIEATQLLMTHPGVSLILATGGAGMVKAAYSSGKPALGVGPGNVPCYIEKTANIKRAVSDLILSKTFDNGTVCASEQAVIIDEEIANEVKKLMREYGCYFLNKEETKKLEEFAIDKNTGLMNPAVVGQPAVKIAQMAGFKVPENTKILVAEYPAVGPKYPLSREKLSPILALYTVKDYKEGIKRCEEMIQFGGLGHSAVIHSENQQIINEFANRVQASRILVNAPASQGAIGDIYNTATPSLTLGCGTMGGNSTTDNVSVYNLINIKRVFIRKERMKWFRVPPQIYFERGSIQYLSQVKGKKAFIVTDPAMVKLGFVDKVTYQLDKANIKYEIFSEVEPDPSVDTVEKGIKIMKEFEPDLLIAVGGGSAIDAAKGMWLFYEYPDTKFEDLRLKFMDIRKRTYRFPELGKKALFIAIPTTSGTGSEVTAFAVITDKKKNIKYPLTDYELTPDIAIIDPDFVMTIPPSVTADTGMDALTHAIEAYVSVMASDYTDALAEKAIKLIFEYLPKAYKNGQDKVAREKMHNASCIAGMAFTNAFLGINHSMAHILGAKFHLPHGRANAILLPYVIEYNAELPKKFASFPQYEYPKAAEKYAEIAKFLGLPASTTDEGVKSLIEAIKNLMKELNLPLTLKDAGINKEEFEKQIMEMADIAFNDQCTGSNPRMPLVSEIAEIYRKAYGE

SEQ ID NO: 11 - DNA, 2619 bp, Thermoanaerobacter ethanolicus
  source 1..2619: mol_type = genomic DNA
atgcctaacttattacaagaaagaagagaagtaaaagaaaaaacagaagtgaaagaaacgctggatgttaaaagacaaatagaccaattagtagaaaaagcacaaagagcacaagaaaaattcatgtcttatacccaagaacaaatagataaaatagttaaagctatggctttggctggtattgaaaatcatgtgagattggcaaaattagcccatgaagaaacaaaaatgggtgtttatgaagacaaaataacgaaaaatctttttgcagtagaatatgtgtacaattatataaaagacaaaaagactgtcggcgtccttagtgaaaacttagaagaaaattatatggaagtggcagaacctgtaggagttatagccggcgtaacacccgttacaaaccctacttctacaacaatgttcaaaagcttaatcgctattaaaacaagaaatccaataatttttagctttcacccaaaagcattaaaatgtagtatagaaacagcaaagaccatgtacgaggcagcattaaaagctggtgcaccagaaggatgcataggttggattgaaacgccttcaattgaagcaacgcaacttctcatgacacatcccggcgtctcccttatcctcgcaacaggcggcgctggaatggtaaaagccgcttacagctcaggaaaacccgcccttggcgtaggtcctggcaatgtcccctgctacattgaaaaaactgcaaatattaaaagagcagtctcagacctaatacttagcaaaacttttgacaatggcacagtatgcgcatcagaacaagctgtgataatagacgaagaaatagcagatgaagtgaaaaaaaatatgaaagaatatggttgctattttctcaataaagaagagactaaaatgctagaagaattcgctatagacaaaaacaccggtttaatgaatccagcagttgtaggtcaaccggcaacaaaaattgctgaaatggctggatttaaagtacctgaaaacacaaaaatacttgtagctgaatatcctgctgtaggaccagaatatcctctctccagagaaaagctaagtccaatacttgctttatacacagtcaaagattacaacgaaggcataaaaagatgtgaagaaatgacagaattcggcggacttggtcactctgcagtaatacattctgaaaaccaacaaattattaatgaatttgcaaaaagagtacgagcaggaagaattcttgtaaacgcccctgcttctcaaggagctattggagatatttataacacggctatcccatctttgactttgggttgcggtacaatgggtagaaattcaacaacagataatgtaagtgtttataaccttataaacataaaacgagtttttataagaaaagagagaatgaaatggttcagagttccaccacaaatttattttgaaagagggtcattacaatatctgtcacaagtaaaaggcaaaaaagcctttattgtaacagaccctgtgatggttaaattaggttttgtagataaagtaacgtatcaattagataaggcaaatattaaatatgaaatattctctgaagttgaaccagatccttcagttgacactgtagaaaaaggggtaaaaataatgagagggtttgagcctgacttactaatagctgtaggtggtggttctgcaatagatgcagcgaagggaatgtggcttttctacgaataccctgatacaaaattcgaagacttaaggttaaaatttatggacataagaaaaagaacttatagatttcctgaactggggaaaaaagctttatttatcgcaataccaaccaccagcggtacaggttctgaagttactgcctttgcagttataacagacaaaaagaaaaatataaagtaccctctcacagattacgaattaacaccagatatcgctataatagaccctgacctcacaatgacaataccaccctctgtcacagcagacactggtatggacgctttaacccatgctattgaagcctatgtatctgtaatggcatcagactatacagacgctctcgcagaaaaagctataaaattgatatttgaatatctacctaaagcatacaaaaacgggcaagataaagtcgcccgcgaaaagatgcacaatgcttcatgcatagctggaatggccttcacaaatgcatttttaggaataaaccatagtatggctcatatacttggtgctaaattccatcttccacacggaagagcaaatgcaatacttctgccctatgtcatagaatacaatgctgagttacctaaaaaatttgcttcattcccacaatatgaatatcccaaagcagccgagaaatatgcagaaattgcaaaattcttgggacttcctgcatcaaccattgaagaaggagtaaaaagcctcattgaagcaataaaaaatcttatgaaagagcttaatcttcctttgacacttaaagaagcaggcataaataaagaagaattcgaaaaacaaataatggaaatgtctgatatagcctttaatgaccagtgcaccggttcaaacccaagaatgccattggtatccgaaattgcagaaatatatagaaaagcctatggagaataa

SEQ ID NO: 12 - protein, 872 aa, Thermoanaerobacter ethanolicus
MPNLLQERREVKEKTEVKETLDVKRQIDQLVEKAQRAQEKFMSYTQEQIDKIVKAMALAGIENHVRLAKLAHEETKMGVYEDKITKNLFAVEYVYNYIKDKKTVGVLSENLEENYMEVAEPVGVIAGVTPVTNPTSTTMFKSLIAIKTRNPIIFSFHPKALKCSIETAKTMYEAALKAGAPEGCIGWIETPSIEATQLLMTHPGVSLILATGGAGMVKAAYSSGKPALGVGPGNVPCYIEKTANIKRAVSDLILSKTFDNGTVCASEQAVIIDEEIADEVKKNMKEYGCYFLNKEETKMLEEFAIDKNTGLMNPAVVGQPATKIAEMAGFKVPENTKILVAEYPAVGPEYPLSREKLSPILALYTVKDYNEGIKRCEEMTEFGGLGHSAVIHSENQQIINEFAKRVRAGRILVNAPASQGAIGDIYNTAIPSLTLGCGTMGRNSTTDNVSVYNLINIKRVFIRKERMKWFRVPPQIYFERGSLQYLSQVKGKKAFIVTDPVMVKLGFVDKVTYQLDKANIKYEIFSEVEPDPSVDTVEKGVKIMRGFEPDLLIAVGGGSAIDAAKGMWLFYEYPDTKFEDLRLKFMDIRKRTYRFPELGKKALFIAIPTTSGTGSEVTAFAVITDKKKNIKYPLTDYELTPDIAIIDPDLTMTIPPSVTADTGMDALTHAIEAYVSVMASDYTDALAEKAIKLIFEYLPKAYKNGQDKVAREKMHNASCIAGMAFTNAFLGINHSMAHILGAKFHLPHGRANAILLPYVIEYNAELPKKFASFPQYEYPKAAEKYAEIAKFLGLPASTIEEGVKSLIEAIKNLMKELNLPLTLKEAGINKEEFEKQIMEMSDIAFNDQCTGSNPRMPLVSEIAEIYRKAYGE

SEQ ID NO: 13 - DNA, 2613 bp, Bacillus coagulans
  source 1..2613: mol_type = genomic DNA
atggcaatcgatgaaaaagttgttggcaaatctgcgcaaatcacggaaatggtcgattccctcgtcgcaaaagggcaaaaagcactgcgtgaatttatggaactggatcaggcacaagtggacaatatcgtaaaacaaatggcacttgccgggttggaacagcatatggtgctcgccaaaatggccgtggaagaaacagggcgcggcgtatatgaagacaaaatgacaaaaaacttgtttgcaacagaatacatctatcacaacattaaatataacaaaacagtcggcatcattgacgaaaacaataatgaagggattgttaaatttgcggaaccggtcggcgtgattgccggggtcactcctgtaacaaacccgacatcaaccacgatgtttaaagcattaattgccattaaaacacgcaacccaattattttcgcgttccatccgtccgcacaaaaatgcagcagccatgccgcaaaagtgatgcttgacgctgctgtgaaagccggcgccccggaaaactgcatccaatggatcgaaaaaccggccattgaagcgacacagcaattgatgaaccattcgggtatttcactgattcttgcaacgggcggttccggcatggtaaagtccgcatattcgagcgggaaacctgcgcttggcgtcgggccgggaaacgtcccttgctatattgaaaaatctgctgatatcaaacgcgccgtcaatgatttgattttgtccaaaacgtttgacaacggcatgatctgtgcgtcggaacaggctgtcatcatcgacaaagaaatttatgacaatgtgaaaaacgaattgattgcaaatcaatgctacttcctgaatgaagcggagaagaaaaaggttgagaaaaccgtcatcaatgaaaagacgcaatccgtcaacagcgccattgtcggcaaaccggcctatgaaattgcgaaaatggcaggcgtaaatgttccggaagataccaaaattttaatcgccgaacttacaggtgtcggcccggactacccgctttccagagaaaaattaagcccggttttggcctgttacaaagccaacagcacaaaacaaggtttcgaatttgcagaagccatgctcgaattcggcggacttggtcactcggctgtgatccattcgacaaacgatgaagtcattgaacaatacggcttaaaaatgaaagccggccggatcattgtcaactccccgtcttcgcaaggggcaatcggcgacatttacaatgcctacatgccttctttgacactcggctgcggcacgtttggcggcaactcggtgtccacaaacgtcggtgtcatcaatctttacaatgtaaaaacaatggcgaaacggagagtcaatatgcaatggtttaaaattccaccgcgcgtgtattttgaaaagaactcggtccaatacctggaaaaaatgccggatatctcaagtgcctttattgtcaccgatccggatatggtcaggcttggattcgttgagaaagtactgtattacttgcggaaacgcccggactatgtgcactgtgaaattttctcagaagtcgaaccggatccgtctattgaaacggttcggaaaggtgccgcagctatggcaagcttccagccggatgtcattatcgcgcttggcggcgggtcggcgatggatgctgcaaaaggcatgtggctgttctatgagcatccggaagttgatttcaacgaattgaagcaaaaatttatggacatccggaaacgggttgccaaattcccgaaactgggtgaaaaagcgcagctggtctgcattccgaccacatcgggcaccggttctgaagtgacttctttcgccgtcatttcggataaaaagaacaacacaaaatatccgctcgcagactatgaactgacaccggatgttgcgatcattgacccgcagtttgttatgaccgttccgaaatccgtaacagccgataccgggatggacgttttgacccatgcgattgaagcctatgtatccaacatggccaacgactatacggacggcctggcaattaaggccatccagcttgttcacgaatacttgccgaaagcatacgcaaatggcaatgatgcactggcacgcgaaaaaatgcacaatgcatcgactttggcagggatggcgttctcgaatgcattccttggcatcaaccattcacttgcccataaaatcggcgctgaattccatattccgcacggccgggctaacgcgattctgttgccgcatgtcatccgctataacgcgcaaaagccgaaaaaatttgcggcattcccgaaatacgaacattttattgcggatcaacgctacgcggaaatcgcgcgcgtacttggtcttccggcaagcacgacagaagaaggtgtcgaaagcctttgccaggaaatcatccggatgtgcaaactgttcaatattccgcttagcctaaaagcagccggcgtgaaccgggcggactttgaaaaacgggttgccattattgcagaccgcgcatttgaagaccaatgcacacctgcaaaccctaaattgccgcttgtcagcgaattggaagacattttacgcaaagcttttgaaggcgttgaagcaaaataa

SEQ ID NO: 14 - protein, 870 aa, Bacillus coagulans
MAIDEKVVGKSAQITEMVDSLVAKGQKALREFMELDQAQVDNIVKQMALAGLEQHMVLAKMAVEETGRGVYEDKMTKNLFATEYIYHNIKYNKTVGIIDENNNEGIVKFAEPVGVIAGVTPVTNPTSTTMFKALIAIKTRNPIIFAFHPSAQKCSSHAAKVMLDAAVKAGAPENCIQWIEKPAIEATQQLMNHSGISLILATGGSGMVKSAYSSGKPALGVGPGNVPCYIEKSADIKRAVNDLILSKTFDNGMICASEQAVIIDKEIYDNVKNELIANQCYFLNEAEKKKVEKTVINEKTQSVNSAIVGKPAYEIAKMAGVNVPEDTKILIAELTGVGPDYPLSREKLSPVLACYKANSTKQGFEFAEAMLEFGGLGHSAVIHSTNDEVIEQYGLKMKAGRIIVNSPSSQGAIGDIYNAYMPSLTLGCGTFGGNSVSTNVGVINLYNVKTMAKRRVNMQWFKIPPRVYFEKNSVQYLEKMPDISSAFIVTDPDMVRLGFVEKVLYYLRKRPDYVHCEIFSEVEPDPSIETVRKGAAAMASFQPDVIIALGGGSAMDAAKGMWLFYEHPEVDFNELKQKFMDIRKRVAKFPKLGEKAQLVCIPTTSGTGSEVTSFAVISDKKNNTKYPLADYELTPDVAIIDPQFVMTVPKSVTADTGMDVLTHAIEAYVSNMANDYTDGLAIKAIQLVHEYLPKAYANGNDALAREKMHNASTLAGMAFSNAFLGINHSLAHKIGAEFHIPHGRANAILLPHVIRYNAQKPKKFAAFPKYEHFIADQRYAEIARVLGLPASTTEEGVESLCQEIIRMCKLFNIPLSLKAAGVNRADFEKRVAIIADRAFEDQCTPANPKLPLVSELEDILRKAFEGVEAK

SEQ ID NO: 15 - DNA, 2604 bp, Geobacillus thermoglucosidasius
  source 1..2604: mol_type = genomic DNA
atggctgtggaggaaagagtcgtcgataaaaaaatcgaagcagcaaaaatgattgatgagcttgtcgctaatgcacagaaagcgttggaacaatttcgcgcttacgatcaagaaacgatcgatcatatcgtgaaagaaatggcgttggccgggctcgacaagcatatggcattagccaagcttgcagtagaagaaacaaaacgtggtgtatatgaagataaaatcataaaaaacctttttgcgacagaatatatataccacaatattaagtacgataaaacagtcgggattattcatgaaaatccgcatgaagaaattatcgaaattgctgagcctgttggtgttattgctgggatcacgccagtgacaaacccgacatcgacgacgatgtttaaagcgttaatctcgataaaaacgcgcaatccgattattttcgctttccatccatcggcacaacgatgcagcagcgaagcggcaagagtgctgcgcgatgcggcggtccgggcaggggctccagaacattgcattcaatggattgaaactccttcgcttgatgcaaccaatcagcttatgcgccatcctggcgtttctctcattttggcaactggtggcgccggcatggtgaaagcagcgtacagctctggaaaaccagctttgggcgtcggacctggaaatgtgccttgctatattgaaaaaacggcaaacataaaacgggcggtaaatgatttaattttatcgaaaacgtttgataacggcatgatttgcgcttctgaacaagcagtcattattgataaagaaatttatgaacaagtaaagaaagaaatgatggaaaaccattgttatttcttaaatgaagaagaaaagaaaaaagtagaaaaactcgttatcaatgaaaatacatgcgccgtcaacccggatatcgtcggaaagccagcttatgaaattgcgaaaatggccggcatcgctgtgccggaagacacaaaaattcttgttgctgagctaaaaggggtcgggccaaaatatccgttgtctcgcgaaaaattaagccctgtccttgcttgctataaagttaacagcacggaagaaggatttaagcgctgtgaagaaatgctggaatttggcggcttgggacattcggctgtcatccattccgataatcaaaacgtggttaccgaatttggcaaacggatgaaagcgggacggattatcgttaatgcgccatcttcgcaaggagcaatcggcgatatttacaatgcgtacattccgtcattaacgctgggatgcggcacatttggcggaaactctgtttcgacaaacgtcagtgcgattcatcttatcaatataaaaagaatggcaaaaaggacggtaaatatgcaatggtttaaagtgccgccgaaaatttatttcgaaaaaaatgctgtacaatacttagcgaaaatgccggatatttccagagcctttatcgtcaccgacccgggaatggtcaagctcggatatgtcgataaagtgctgtattacttgcgcagacgcccggattatgtgcatagtgaaattttctccgaagtagagccagatccttcaattgagacggtaatgaaaggcgtcgacatgatgagaagtttcgagccggatgtgattatcgcgctcggaggcggctcgccaatggatgcggcaaaagcgatgtggctcttttacgagcatccgacagcggatttcaacgcattaaaacaaaaatttttagatattcgaaaacgcgtttataaatatccaaaactgggccaaaaagcgaaatttgtcgccattccgacgacatcaggaacaggatcggaagtaacgtcctttgccgtcattaccgataaaaaaacgaatataaaatatccgttggcagattatgaattgacaccggacgtcgcgattgtggatccgcaatttgtcatgacagtgccaaaacatgtcaccgccgatacgggaatggatgtattgacacatgcgatcgaagcgtatgtctccaatatggccaatgattataccgatggtcttgccatgaaagcaatccaactcgtatttgaatatttgccgcgggcatatcaaaacggagcggatgagcttgcccgggagaaaatgcataacgcctctacgattgcgggaatggcatttgccaacgcgtttttaggcattaaccatagtttggctcataaacttggcgcggaattccatattccgcatgggcgcgcgaataccattttgatgccgcatgtcattcgctataacgcagcgaaaccgaaaaaatttaccgcatttccgaaatacgaatatttcaaagcggaccagcgctatgcagaaattgcgagaatgctcggcttgccggcccgcacaacggaagaaggggtcgaaagcctcgttcaggcgatcattaagctggcaaaacagttggatatgccgctgagcattgaagcatgcggcgtcagcaaacaagaatttgaaagcaaagttgaaaaattagccgaattggctttcgaagaccaatgtactactgctaacccgaaactcccgcttgttagcgatttagttcatatttatcgccaagcgtttaaaggagtttaa

SEQ ID NO: 16 - protein, 867 aa, Geobacillus thermoglucosidasius
MAVEERVVDKKIEAAKMIDELVANAQKALEQFRAYDQETIDHIVKEMALAGLDKHMALAKLAVEETKRGVYEDKIIKNLFATEYIYHNIKYDKTVGIIHENPHEEIIEIAEPVGVIAGITPVTNPTSTTMFKALISIKTRNPIIFAFHPSAQRCSSEAARVLRDAAVRAGAPEHCIQWIETPSLDATNQLMRHPGVSLILATGGAGMVKAAYSSGKPALGVGPGNVPCYIEKTANIKRAVNDLILSKTFDNGMICASEQAVIIDKEIYEQVKKEMMENHCYFLNEEEKKKVEKLVINENTCAVNPDIVGKPAYEIAKMAGIAVPEDTKILVAELKGVGPKYPLSREKLSPVLACYKVNSTEEGFKRCEEMLEFGGLGHSAVIHSDNQNVVTEFGKRMKAGRIIVNAPSSQGAIGDIYNAYIPSLTLGCGTFGGNSVSTNVSAIHLINIKRMAKRTVNMQWFKVPPKIYFEKNAVQYLAKMPDISRAFIVTDPGMVKLGYVDKVLYYLRRRPDYVHSEIFSEVEPDPSIETVMKGVDMMRSFEPDVIIALGGGSPMDAAKAMWLFYEHPTADFNALKQKFLDIRKRVYKYPKLGQKAKFVAIPTTSGTGSEVTSFAVITDKKTNIKYPLADYELTPDVAIVDPQFVMTVPKHVTADTGMDVLTHAIEAYVSNMANDYTDGLAMKAIQLVFEYLPRAYQNGADELAREKMHNASTIAGMAFANAFLGINHSLAHKLGAEFHIPHGRANTILMPHVIRYNAAKPKKFTAFPKYEYFKADQRYAEIARMLGLPARTTEEGVESLVQAIIKLAKQLDMPLSIEACGVSKQEFESKVEKLAELAFEDQCTTANPKLPLVSDLVHIYRQAFKGV

SEQ ID NO: 17 - DNA, 2613 bp, Fonticella tunisiensis
  source 1..2613: mol_type = genomic DNA
atgaaagtaacaaatgcagaagaactaagattaaagcttgaggaggttagaaaagcccaaaaaatattcgcctcctacacccaggaacaggtagatgaaatatttagacaggctgctatggctgctaacaatgcaagaattaagcttgcaaagatggctgttgaagaaacaggaatgggaattgtagaagacaaagttattaaaaaccactttgcctcagaatatatatacaataaatataaggatgaaaagacctgcggagttattgacagagatgaatccttcggcataatgagggttgcagaacctataggagttatcgctgcaatagtaccaactaccaacccgacatccactgcaatatttaaagcattaatcgctttaaaaacaagaaacggtgtgattttctcaccccatccaagggctaaaaaatcaactatagcagcagctaaaatcgtacttgatgctgcagttaaggccggtgcccctgagggaataataggatggattgatgaaccaacggttgaactttcacagatcgttatgaaggaagctgatatgatacttgccacaggcggccccggaatggtaagagctgcttattcctcaggaaaacccgcaataggagtaggtgctggaaatacgcctgcaataatagatgaaacagcacatattaaaatggcagtaagctccatacttctttcaaagacatttgacaacggagttatatgtgcttcagaacagtcagtaattgtaatggaacaaatatatgacgaagttaagcgtgagtttgaggaaagaggagcatacttcctaaagggagaggaaatcgacaaggttagaaagataatacttgttaatggttcaataaatgcaaatatagttggacagcctgcccacaaaatagctgaaatggctggagttaaagttcctgaaacagcaaaggtattaatcggagaagttgaatccgttgaactcgatgaaccattctcacacgaaaaactttcacctgtgctcgctatgtataaggctaaaaccttcgatgaggcacttcagaaagctgcaaggcttgtggaacttggcggatttgggcatacatcagttctatataccgaccaggtaaaatcaagggatagaattgaaaaatttggtgcgactatgaagacaggaagaacaataatcaatatgccttcgtcccaaggtgcaataggagatatctataacttcaggcttgctccttcgctaacactcggatgtggtacatggggtggaaactctgtatctgaaaacgttggagttaagcatcttttaaacatcaagagtgttgctgaaaggagagaaaatatgctttggttcagagttcctgaaaagatatacttcaaatacggctgcctgcctgtagcattaaaggaattaaaggatatgggcaagaagagggcattcatcgttactgacaaagttctgtataatttaggatttatcgatacagttacaaagacccttgatgaaataggaattgaatatagcgtgttctttgacgttgaaccagacccaacacttgcaactgcaagaaagggtgcagcacaaatgaaaagcctcaatccggatgtaataattgcagttggtggaggctcacctatggatgctgcaaagattatgtgggtactttatgagcatccggaagtaaggtttgaagaccttgcaatgagatttatggatattagaaagagagtttaccagttcccaaagatgggcgaaaaggctatgatggtttcaatcccaacttcttccggaacaggttcagaggttactccatttgctgttataaccgatgaaaagacgggaattaaatatcctcttgcagactatgagttaactcctgatatggcaatagtagatgcagaacttatgctcaatatgccaaagggacttacagcagcatctggtatagacgccctaactcatgcaatagaagcctatgtttcggtacttgcatcagagtatactaacggacttgcccttgaagcgataagacttatattcaaatatctaccacaggcatataatgatggtccaaacaacatcaaagcaagggaaaagatggcccacgctgcaactatggctggtatggcctttgcaaatgcattcctcggcgtatgccactcaatggcccacaagcttggagcaatgcatcatgtaccacacggagttgccaacggccttctaattaacgaagtaataagatttaatgcagttgataacccaagaaagcaaactgcattcccacagtataaatatccaaacgccaagttcagatatgcaaggattgctgactacctgaaccttggcggaaataccgaagatgaaaagattgaactccttataaaggcaatcgacgacttaaagaaccaggttaacatgccaaaaacgataagtgaagctggtgtttcaagagagaaattctacgcaacccttgatgaaatgtgcgaacaggccttcgacgaccagtgcacaggtgccaacccaagatatccgttaataagcgaaatcaagcagatgtatataaacgctttcgaaggaatttcaaaggaaactgaagaaaataataaataa

SEQ ID NO: 18 - protein, 870 aa, Fonticella tunisiensis
MKVTNAEELRLKLEEVRKAQKIFASYTQEQVDEIFRQAAMAANNARIKLAKMAVEETGMGIVEDKVIKNHFASEYIYNKYKDEKTCGVIDRDESFGIMRVAEPIGVIAAIVPTTNPTSTAIFKALIALKTRNGVIFSPHPRAKKSTIAAAKIVLDAAVKAGAPEGIIGWIDEPTVELSQIVMKEADMILATGGPGMVRAAYSSGKPAIGVGAGNTPAIIDETAHIKMAVSSILLSKTFDNGVICASEQSVIVMEQIYDEVKREFEERGAYFLKGEEIDKVRKIILVNGSINANIVGQPAHKIAEMAGVKVPETAKVLIGEVESVELDEPFSHEKLSPVLAMYKAKTFDEALQKAARLVELGGFGHTSVLYTDQVKSRDRIEKFGATMKTGRTIINMPSSQGAIGDIYNFRLAPSLTLGCGTWGGNSVSENVGVKHLLNIKSVAERRENMLWFRVPEKIYFKYGCLPVALKELKDMGKKRAFIVTDKVLYNLGFIDTVTKTLDEIGIEYSVFFDVEPDPTLATARKGAAQMKSLNPDVIIAVGGGSPMDAAKIMWVLYEHPEVRFEDLAMRFMDIRKRVYQFPKMGEKAMMVSIPTSSGTGSEVTPFAVITDEKTGIKYPLADYELTPDMAIVDAELMLNMPKGLTAASGIDALTHAIEAYVSVLASEYTNGLALEAIRLIFKYLPQAYNDGPNNIKAREKMAHAATMAGMAFANAFLGVCHSMAHKLGAMHHVPHGVANGLLINEVIRFNAVDNPRKQTAFPQYKYPNAKFRYARIADYLNLGGNTEDEKIELLIKAIDDLKNQVNMPKTISEAGVSREKFYATLDEMCEQAFDDQCTGANPRYPLISEIKQMYINAFEGISKETEENNK

SEQ ID NO: 19 - DNA, 35 bp, synthetic construct
  source 1..35: mol_type = other DNA
ttttataacccgggccatcgactgcacggtgcacc

SEQ ID NO: 20 - DNA, 35 bp, synthetic construct
  source 1..35: mol_type = other DNA
tgctagcactgtttcctgtgtgaaattgttatccg

SEQ ID NO: 21 - DNA, 38 bp, synthetic construct
  source 1..38: mol_type = other DNA
ggaaacagtgctagcagatctggaggagaaacgcatat

SEQ ID NO: 22 - DNA, 72 bp, synthetic construct
  source 1..72: mol_type = other DNA
cagtgcggccgcaagcttgtcgacggagctcgaattcggatccgatatcagcatatgcgtttctcctccaga

SEQ ID NO: 23 - DNA, 80 bp, synthetic construct
  source 1..80: mol_type = other DNA
acaagcttgcggccgcactgcagcaccatcaccaccatcattgataagatccggctgctaacaaagcccgaaaggaagct

SEQ ID NO: 24 - DNA, 63 bp, synthetic construct
  source 1..63: mol_type = other DNA
tatttgaatcgagttattgctcagcggtggcagcagccaactcagcttcctttcgggctttgt

SEQ ID NO: 25 - DNA, 35 bp, synthetic construct
  source 1..35: mol_type = other DNA
taactcgattcaaataaaacgaaaggctcagtcga

SEQ ID NO: 26 - DNA, 35 bp, synthetic construct
  source 1..35: mol_type = other DNA
cctagatccgcggagtttgtagaaacgcaaaaagg

SEQ ID NO: 27 - DNA, 35 bp, synthetic construct
  source 1..35: mol_type = other DNA
acaaactccgcggatctaggtgaagatcctttttg

SEQ ID NO: 28 - DNA, 35 bp, synthetic construct
  source 1..35: mol_type = other DNA
cgtccgcggccagcaaaaggccaggaaccgtaaaa

SEQ ID NO: 29 - DNA, 35 bp, synthetic construct
  source 1..35: mol_type = other DNA
ttgctggccgcggacgtagaaagcctgtccgcaga

SEQ ID NO: 30 - DNA, 35 bp, synthetic construct
  source 1..35: mol_type = other DNA
ggcccgggttataaaagccagtcattaggcctatc

SEQ ID NO: 31 - DNA, 35 bp, synthetic construct
  source 1..35: mol_type = other DNA
aattgtcagataggcctaatgactggcttttataa

SEQ ID NO: 32 - DNA, 35 bp, synthetic construct
  source 1..35: mol_type = other DNA
tgacgccagaagcattggtgcaccgtgcagtcgat

SEQ ID NO: 33 - DNA, 19 bp, synthetic construct
  source 1..19: mol_type = other DNA
gatctggaggagaaacgca

SEQ ID NO: 34 - DNA, 17 bp, synthetic construct
  source 1..17: mol_type = other DNA
tatgcgtttctcctcca

SEQ ID NO: 35 - DNA, 35 bp, synthetic construct
  source 1..35: mol_type = other DNA
gaggccatctaggccatgagtaagtctgacggaac

SEQ ID NO: 36 - DNA, 35 bp, synthetic construct
  source 1..35: mol_type = other DNA
atccggcacccatatctgaaccggacgcaaacccg

SEQ ID NO: 37 - DNA, 35 bp, synthetic construct
  source 1..35: mol_type = other DNA
ttcagatatgggtgccggatacccgccgcccgggc

SEQ ID NO: 38 - DNA, 35 bp, synthetic construct
  source 1..35: mol_type = other DNA
aaggccttcatggccttatttcgcgattcccaaga

SEQ ID NO: 39 - DNA, 44 bp, synthetic construct
  source 1..44: mol_type = other DNA
gatctggaggagaaacgcatatgaaagtaacaaacatagaagag

SEQ ID NO: 40 - DNA, 47 bp, synthetic construct
  source 1..47: mol_type = other DNA
tgtcgacggagctcgaattcttatttttctcccattttaatttcacc

SEQ ID NO: 41 - DNA, 44 bp, synthetic construct
  source 1..44: mol_type = other DNA
gatctggaggagaaacgcatatgagagcagcagtcgtcagttct

SEQ ID NO: 42 - DNA, 44 bp, synthetic construct
  source 1..44: mol_type = other DNA
tgtcgacggagctcgaattcttatttcaacgacatatccaggac

SEQ ID NO: 43 - DNA, 44 bp, synthetic construct
  source 1..44: mol_type = other DNA
gatctggaggagaaacgcatatgaaagcagccgtcataactaaa

SEQ ID NO: 44 - DNA, 44 bp, synthetic construct
  source 1..44: mol_type = other DNA
tgtcgacggagctcgaattcctagtgatgggtaaaatcaacaac

SEQ ID NO: 45 - DNA, 44 bp, synthetic construct
  source 1..44: mol_type = other DNA
gatctggaggagaaacgcatatggaaaacaaagaaagaaagatt

SEQ ID NO: 46 - DNA, 44 bp, synthetic construct
  source 1..44: mol_type = other DNA
tgtcgacggagctcgaattctcatgctctcttcgctccgactct

SEQ ID NO: 47 - DNA, 44 bp, synthetic construct
  source 1..44: mol_type = other DNA
gatctggaggagaaacgcatatgcctactttattacaagaaaaa

SEQ ID NO: 48 - DNA, 44 bp, synthetic construct
  source 1..44: mol_type = other DNA
tgtcgacggagctcgaattcttattctccataggcttttctata

SEQ ID NO: 49 - DNA, 44 bp, synthetic construct
  source 1..44: mol_type = other DNA
gatctggaggagaaacgcatatgcctaacttattacaagaaaga

SEQ ID NO: 50 - DNA, 44 bp, synthetic construct; identical to SEQ ID NO: 48
  source 1..44: mol_type = other DNA

SEQ ID NO: 51 - DNA, 44 bp, synthetic construct
  source 1..44: mol_type = other DNA
gatctggaggagaaacgcatatggcaatcgatgaaaaagttgtt

SEQ ID NO: 52 - DNA, 44 bp, synthetic construct
  source 1..44: mol_type = other DNA
tgtcgacggagctcgaattcttattttgcttcaacgccttcaaa

SEQ ID NO: 53 - DNA, 44 bp, synthetic construct
  source 1..44: mol_type = other DNA
gatctggaggagaaacgcatatggctgtggaggaaagagtcgtc

SEQ ID NO: 54 - DNA, 44 bp, synthetic construct
  source 1..44: mol_type = other DNA
tgtcgacggagctcgaattcttaaactcctttaaacgcttggcg

SEQ ID NO: 55 - DNA, 44 bp, synthetic construct
  source 1..44: mol_type = other DNA
gatctggaggagaaacgcatatgagggttgcagaacctatagga

SEQ ID NO: 56 - DNA, 44 bp, synthetic construct
  source 1..44: mol_type = other DNA
tgtcgacggagctcgaattcttatttattattttcttcagtttc

SEQ ID NO: 57 - DNA, 20 bp, synthetic construct
  source 1..20: mol_type = other DNA
gaattcgagctccgtcgaca

SEQ ID NO: 58 - DNA, 20 bp, synthetic construct
  source 1..20: mol_type = other DNA
atgcgtttctcctccagatc